European Patent Application EP 4 269 422 A1, published November 1, 2023. Title: METHOD FOR PREPARING PEPTIDE COMPOUNDS CONTAINING N-SUBSTITED AMINO ACID RESIDUE. Applicant: CHUGAI SEIYAKU KABUSHIKI KAISHA. The sequence listing filed with the application follows.

SEQUENCE LISTING (39 sequences)

SEQ ID NO: 1 - protein, 5 aa, Artificial Sequence
  An artificially synthesized sequence
  MISC_FEATURE (1)..(1): Fmoc-MeAla
  MISC_FEATURE (2)..(2): MeLeu
  MISC_FEATURE (4)..(4): MeVal
  MISC_FEATURE (5)..(5): MeAsp-pip
XXAXX

SEQ ID NO: 2 - protein, 5 aa, Artificial Sequence
  An artificially synthesized sequence
  MISC_FEATURE (1)..(1): Fmoc-MeAla
  MISC_FEATURE (2)..(2): MeLeu
  MISC_FEATURE (4)..(4): MeVal
  MISC_FEATURE (5)..(5): Asp-NMe2
XXGXX

SEQ ID NO: 3 - protein, 5 aa, Artificial Sequence
  An artificially synthesized sequence
  MISC_FEATURE (1)..(1): Fmoc-MeAla
  MISC_FEATURE (2)..(2): MeLeu
  MISC_FEATURE (4)..(4): bAla(2-Me2)
  MISC_FEATURE (5)..(5): D-3-MeAbu-OH
XXGXX

SEQ ID NO: 4 - protein, 5 aa, Artificial Sequence
  An artificially synthesized sequence
  MISC_FEATURE (1)..(1): Fmoc-MeAla
  MISC_FEATURE (3)..(3): MeAla
  MISC_FEATURE (5)..(5): Pro-OH
XLXFX

SEQ ID NO: 5 - protein, 7 aa, Artificial Sequence
  An artificially synthesized sequence
  MISC_FEATURE (1)..(1): Fmoc-MeAla
  MISC_FEATURE (3)..(3): MeGly
  MISC_FEATURE (4)..(4): MeAla
  MISC_FEATURE (6)..(6): MeGly(cPent)
  MISC_FEATURE (7)..(7): MeAsp-NMe2
XLXXAXX

SEQ ID NO: 6 - protein, 7 aa, Artificial Sequence
  An artificially synthesized sequence
  MISC_FEATURE (1)..(1): Fmoc-MeAla
  MISC_FEATURE (3)..(3): MeLeu
  MISC_FEATURE (4)..(4): MeAla
  MISC_FEATURE (6)..(6): Aib
  MISC_FEATURE (7)..(7): MeAsp-NMe2
XLXXGXX

SEQ ID NO: 7 - protein, 7 aa, Artificial Sequence
  An artificially synthesized sequence
  MISC_FEATURE (1)..(1): Fmoc-MeAla
  MISC_FEATURE (3)..(3): MeGly
  MISC_FEATURE (4)..(4): MeAla
  MISC_FEATURE (6)..(6): MeVal
  MISC_FEATURE (7)..(7): Gly-OH
XLXXAXX

SEQ ID NO: 8 - protein, 7 aa, Artificial Sequence
  An artificially synthesized sequence
  MISC_FEATURE (1)..(1): Fmoc-MeAla
  MISC_FEATURE (3)..(3): MeLeu
  MISC_FEATURE (5)..(5): MeAla
  MISC_FEATURE (7)..(7): Tyr(tBu)-OH
XLXAXGX

SEQ ID NO: 9 - protein, 9 aa, Artificial Sequence
  An artificially synthesized sequence
  MISC_FEATURE (1)..(1): Fmoc-MeAla
  MISC_FEATURE (3)..(3): MeGly
  MISC_FEATURE (4)..(4): MeAla
  MISC_FEATURE (6)..(6): MePhe
  MISC_FEATURE (8)..(8): MeChg
  MISC_FEATURE (9)..(9): D-3-MeAbu-OH
XLXXLXAXX

SEQ ID NO: 10 - protein, 9 aa, Artificial Sequence
  An artificially synthesized sequence
  MISC_FEATURE (1)..(1): Fmoc-MeAla
  MISC_FEATURE (3)..(3): MeLeu
  MISC_FEATURE (5)..(5): MePhe
  MISC_FEATURE (7)..(7): MeLeu
  MISC_FEATURE (9)..(9): MeAsp-NMe2
XLXAXAXGX

SEQ ID NO: 11 - protein, 9 aa, Artificial Sequence
  An artificially synthesized sequence
  MISC_FEATURE (1)..(1): Fmoc-MeAla
  MISC_FEATURE (3)..(3): MeGly
  MISC_FEATURE (4)..(4): MeAla
  MISC_FEATURE (6)..(6): MePhe
  MISC_FEATURE (8)..(8): MeVal
  MISC_FEATURE (9)..(9): Pro-OH
XLXXLXAXX

SEQ ID NO: 12 - protein, 9 aa, Artificial Sequence
  An artificially synthesized sequence
  MISC_FEATURE (1)..(1): Fmoc-MeAla
  MISC_FEATURE (3)..(3): MeLeu
  MISC_FEATURE (5)..(5): MePhe
  MISC_FEATURE (7)..(7): MeLeu
  MISC_FEATURE (9)..(9): Ala-OH
XLXAXGXAX

SEQ ID NO: 13 - protein, 11 aa, Artificial Sequence
  An artificially synthesized sequence
  MISC_FEATURE (1)..(1): Fmoc-MeAla
  MISC_FEATURE (3)..(3): MeGly
  MISC_FEATURE (6)..(6): MePhe
  MISC_FEATURE (10)..(10): MeLeu
  MISC_FEATURE (11)..(11): MeAsp-pip
XLXALXAPAXX

SEQ ID NO: 14 - protein, 11 aa, Artificial Sequence
  An artificially synthesized sequence
  MISC_FEATURE (1)..(1): Fmoc-MeAla
  MISC_FEATURE (3)..(3): MeLeu
  MISC_FEATURE (6)..(6): MePhe
  MISC_FEATURE (7)..(7): MeAla
  MISC_FEATURE (10)..(10): D-MeVal
  MISC_FEATURE (11)..(11): MeAsp-NMe2
XLXAGXXLGXX

SEQ ID NO: 15 - protein, 11 aa, Artificial Sequence
  An artificially synthesized sequence
  MISC_FEATURE (1)..(1): Fmoc-MeAla
  MISC_FEATURE (3)..(3): MeGly
  MISC_FEATURE (6)..(6): MePhe
  MISC_FEATURE (9)..(9): MeAla
  MISC_FEATURE (10)..(10): Lys(Boc)
  MISC_FEATURE (11)..(11): Pro-OH
XLXALXAPXXX

SEQ ID NO: 16 - protein, 11 aa, Artificial Sequence
  An artificially synthesized sequence
  MISC_FEATURE (1)..(1): Fmoc-MeAla
  MISC_FEATURE (3)..(3): MeLeu
  MISC_FEATURE (6)..(6): MePhe
  MISC_FEATURE (7)..(7): MeAla
  MISC_FEATURE (9)..(9): MeAla
  MISC_FEATURE (11)..(11): Gly-OH
XLXAGXXLXFX

SEQ ID NO: 17 - protein, 13 aa, Artificial Sequence
  An artificially synthesized sequence
  MISC_FEATURE (1)..(1): Fmoc-MeAla
  MISC_FEATURE (3)..(3): MeGly
  MISC_FEATURE (4)..(4): MeAla
  MISC_FEATURE (6)..(6): MePhe
  MISC_FEATURE (7)..(7): MeAla
  MISC_FEATURE (10)..(10): MeLeu
  MISC_FEATURE (12)..(12): MeChg
  MISC_FEATURE (13)..(13): MeAsp-pip
XLXXLXXGLXAXX

SEQ ID NO: 18 - protein, 13 aa, Artificial Sequence
  An artificially synthesized sequence
  MISC_FEATURE (1)..(1): Fmoc-MeAla
  MISC_FEATURE (3)..(3): MeLeu
  MISC_FEATURE (5)..(5): MePhe
  MISC_FEATURE (7)..(7): MeAla
  MISC_FEATURE (10)..(10): MeLeu
  MISC_FEATURE (12)..(12): bAla(2-Me2)
  MISC_FEATURE (13)..(13): MeAsp-NMe2
XLXAXGXLAXGXX

SEQ ID NO: 19 - protein, 13 aa, Artificial Sequence
  An artificially synthesized sequence
  MISC_FEATURE (1)..(1): Fmoc-MeAla
  MISC_FEATURE (3)..(3): MeGly
  MISC_FEATURE (4)..(4): MeAla
  MISC_FEATURE (6)..(6): MePhe
  MISC_FEATURE (7)..(7): MeAla
  MISC_FEATURE (10)..(10): MeLeu
  MISC_FEATURE (12)..(12): MeLeu
  MISC_FEATURE (13)..(13): Aib-OH
XLXXLXXGLXAXX

SEQ ID NO: 20 - protein, 13 aa, Artificial Sequence
  An artificially synthesized sequence
  MISC_FEATURE (1)..(1): Fmoc-MeAla
  MISC_FEATURE (3)..(3): MeLeu
  MISC_FEATURE (5)..(5): MePhe
  MISC_FEATURE (7)..(7): MeAla
  MISC_FEATURE (10)..(10): MeLeu
  MISC_FEATURE (11)..(11): MeAla
  MISC_FEATURE (12)..(12): Asn(Trt)
  MISC_FEATURE (13)..(13): Gly-OH
XLXAXGXLAXXXX

SEQ ID NO: 21 - protein, 15 aa, Artificial Sequence
  An artificially synthesized sequence
  MISC_FEATURE (1)..(1): Fmoc-MeAla
  MISC_FEATURE (3)..(3): MeGly
  MISC_FEATURE (6)..(6): MePhe
  MISC_FEATURE (7)..(7): MeAla
  MISC_FEATURE (9)..(9): MePhe
  MISC_FEATURE (12)..(12): MeLeu
  MISC_FEATURE (14)..(14): MeVal
  MISC_FEATURE (15)..(15): D-MeAsp-NMe2
XLXALXXGXPAXGXX

SEQ ID NO: 22 - protein, 15 aa, Artificial Sequence
  An artificially synthesized sequence
  MISC_FEATURE (1)..(1): Fmoc-MeAla
  MISC_FEATURE (3)..(3): MeLeu
  MISC_FEATURE (5)..(5): MePhe
  MISC_FEATURE (7)..(7): MeAla
  MISC_FEATURE (9)..(9): MePhe
  MISC_FEATURE (10)..(10): MeAla
  MISC_FEATURE (12)..(12): MeLeu
  MISC_FEATURE (14)..(14): MeVal
  MISC_FEATURE (15)..(15): MeGly-OH
XLXAXGXLXXAXAXX

SEQ ID NO: 23 - protein, 15 aa, Artificial Sequence
  An artificially synthesized sequence
  MISC_FEATURE (1)..(1): Fmoc-MeAla
  MISC_FEATURE (3)..(3): MeGly
  MISC_FEATURE (6)..(6): MePhe
  MISC_FEATURE (7)..(7): MeAla
  MISC_FEATURE (9)..(9): MePhe
  MISC_FEATURE (10)..(10): MeAla
  MISC_FEATURE (12)..(12): MeLeu
  MISC_FEATURE (13)..(13): MeAla
  MISC_FEATURE (15)..(15): Val-OH
XLXALXXGXXAXXGX

SEQ ID NO: 24 - protein, 15 aa, Artificial Sequence
  An artificially synthesized sequence
  MISC_FEATURE (1)..(1): Fmoc-MeAla
  MISC_FEATURE (3)..(3): MeLeu
  MISC_FEATURE (5)..(5): MePhe
  MISC_FEATURE (7)..(7): MeAla
  MISC_FEATURE (9)..(9): MePhe
  MISC_FEATURE (12)..(12): MeLeu
  MISC_FEATURE (13)..(13): MeAla
  MISC_FEATURE (14)..(14): Ser(tBu)
  MISC_FEATURE (15)..(15): Gly-OH
XLXAXGXLXPAXXXX

SEQ ID NO: 25 - protein, 6 aa, Artificial Sequence
  An artificially synthesized sequence
  MISC_FEATURE (1)..(1): Fmoc-MeAla
  MISC_FEATURE (3)..(3): MeLeu
  MISC_FEATURE (6)..(6): Pro-OH
XLXAAX

SEQ ID NO: 26 - protein, 6 aa, Artificial Sequence
  An artificially synthesized sequence
  MISC_FEATURE (1)..(1): Fmoc-MeAla
  MISC_FEATURE (3)..(3): MeLeu
  MISC_FEATURE (5)..(5): MeGly(cPent)
  MISC_FEATURE (6)..(6): MeAsp-NMe2
XLXAXX

SEQ ID NO: 27 - protein, 10 aa, Artificial Sequence
  An artificially synthesized sequence
  MISC_FEATURE (1)..(1): Fmoc-MeAla
  MISC_FEATURE (2)..(2): MeLeu
  MISC_FEATURE (4)..(4): MeGly
  MISC_FEATURE (5)..(5): MePhe
  MISC_FEATURE (7)..(7): MeLeu
  MISC_FEATURE (10)..(10): Pro-OH
XXAXXLXAAX

SEQ ID NO: 28 - protein, 10 aa, Artificial Sequence
  An artificially synthesized sequence
  MISC_FEATURE (1)..(1): Fmoc-MeAla
  MISC_FEATURE (2)..(2): MeLeu
  MISC_FEATURE (4)..(4): MeLeu
  MISC_FEATURE (5)..(5): MePhe
  MISC_FEATURE (7)..(7): MeAla
  MISC_FEATURE (9)..(9): MeGly(cPent)
  MISC_FEATURE (10)..(10): MeAsp-NMe2
XXAXXLXAXX

SEQ ID NO: 29 - protein, 14 aa, Artificial Sequence
  An artificially synthesized sequence
  MISC_FEATURE (1)..(1): Fmoc-MeAla
  MISC_FEATURE (3)..(3): MeGly
  MISC_FEATURE (4)..(4): MeAla
  MISC_FEATURE (6)..(6): MePhe
  MISC_FEATURE (7)..(7): MeAla
  MISC_FEATURE (10)..(10): MeLeu
  MISC_FEATURE (11)..(11): MeAla
  MISC_FEATURE (14)..(14): Pro-OH
XLXXLXXGLXXAAX

SEQ ID NO: 30 - protein, 14 aa, Artificial Sequence
  An artificially synthesized sequence
  MISC_FEATURE (1)..(1): Fmoc-MeAla
  MISC_FEATURE (3)..(3): MeGly
  MISC_FEATURE (4)..(4): MeAla
  MISC_FEATURE (6)..(6): MePhe
  MISC_FEATURE (7)..(7): MeAla
  MISC_FEATURE (10)..(10): MeLeu
  MISC_FEATURE (11)..(11): MeAla
  MISC_FEATURE (13)..(13): MeGly(cPent)
  MISC_FEATURE (14)..(14): MeAsp-NMe2
XLXXLXXGLXXAXX

SEQ ID NO: 31 - protein, 5 aa, Artificial Sequence
  An artificially synthesized sequence
  MISC_FEATURE (1)..(1): Fmoc-MeAla
  MISC_FEATURE (4)..(4): MeVal
  MISC_FEATURE (5)..(5): MeAsn-pip
XLAXX

SEQ ID NO: 32 - protein, 7 aa, Artificial Sequence
  An artificially synthesized sequence
  MISC_FEATURE (1)..(1): Fmoc-MeAla
  MISC_FEATURE (3)..(3): MeGly
  MISC_FEATURE (4)..(4): MeAla
  MISC_FEATURE (6)..(6): MeVal
  MISC_FEATURE (7)..(7): MeAsn-pip
XLXXAXX

SEQ ID NO: 33 - protein, 11 aa, Artificial Sequence
  An artificially synthesized sequence
  MISC_FEATURE (1)..(1): Fmoc-MeAla
  MISC_FEATURE (3)..(3): MeGly
  MISC_FEATURE (6)..(6): MePhe
  MISC_FEATURE (10)..(10): MeVal
  MISC_FEATURE (11)..(11): MeAsn-pip
XLXALXAPAXX

SEQ ID NO: 34 - protein, 11 aa, Artificial Sequence
  An artificially synthesized sequence
  MISC_FEATURE (1)..(1): H-MeAla
  MISC_FEATURE (3)..(3): MeGly
  MISC_FEATURE (5)..(5): MePhe
  MISC_FEATURE (7)..(7): MeAla
  MISC_FEATURE (10)..(10): MeVal
  MISC_FEATURE (11)..(11): MeAsp-pip
XLXAXLXLGXX

SEQ ID NO: 35 - protein, 11 aa, Artificial Sequence
  An artificially synthesized sequence
  MISC_FEATURE (1)..(1): H-MeAla
  MISC_FEATURE (3)..(3): MeLeu
  MISC_FEATURE (5)..(5): MePhe
  MISC_FEATURE (7)..(7): MeAla
  MISC_FEATURE (10)..(10): MeVal
  MISC_FEATURE (11)..(11): Asp-NMe2
XLXAXGXLAXX

SEQ ID NO: 36 - protein, 11 aa, Artificial Sequence
  An artificially synthesized sequence
  MISC_FEATURE (1)..(1): H-MeAla
  MISC_FEATURE (5)..(5): MePhe
  MISC_FEATURE (7)..(7): MeAla
  MISC_FEATURE (8)..(8): MeLeu
  MISC_FEATURE (10)..(10): MeVal
  MISC_FEATURE (11)..(11): MeGly-OH
XLPAXLXXAXX

SEQ ID NO: 37 - protein, 11 aa, Artificial Sequence
  An artificially synthesized sequence
  MISC_FEATURE (1)..(1): H-MeAla
  MISC_FEATURE (2)..(2): MeLeu
  MISC_FEATURE (4)..(4): MeAla
  MISC_FEATURE (5)..(5): MePhe
  MISC_FEATURE (7)..(7): MeLeu
  MISC_FEATURE (9)..(9): MeAla
  MISC_FEATURE (11)..(11): Gly-OH
XXGXXAXLXFX

SEQ ID NO: 38 - protein, 12 aa, Artificial Sequence
  An artificially synthesized sequence
  MISC_FEATURE (1)..(1): H-MeAla
  MISC_FEATURE (3)..(3): MeGly
  MISC_FEATURE (5)..(5): MePhe
  MISC_FEATURE (7)..(7): MeAla
  MISC_FEATURE (9)..(9): MeLeu
  MISC_FEATURE (12)..(12): Pro-OH
XLXAXLXLXAAX

SEQ ID NO: 39 - protein, 12 aa, Artificial Sequence
  An artificially synthesized sequence
  MISC_FEATURE (1)..(1): H-MeAla
  MISC_FEATURE (3)..(3): MeLeu
  MISC_FEATURE (5)..(5): MePhe
  MISC_FEATURE (7)..(7): MeAla
  MISC_FEATURE (9)..(9): MeAla
  MISC_FEATURE (11)..(11): MeGly(cPent)
  MISC_FEATURE (12)..(12): MeAsp-NMe2
XLXAXGXLXAXX